European Patent Application EP 4 223 881 A1, published August 9, 2023. Title: METHOD AND SYSTEM FOR DELIVERING NUCLEIC ACID. Applicant: Shanghai Ranai Marketing Consulting Partnaership(Limited Partnership). The sequence listing filed with the application follows.

SEQUENCE LISTING (7 sequences)

SEQ ID NO: 1 - DNA, 1610 bp, Artificial Sequence
  2 Ambystoma laterale x Ambystoma jeffersonianum
ccatgcattagttattaatagtaatcaattacggggtcattagttcatagcccatatatggagttccgcgttacataacttacggtaaatggcccgcctggctgaccgcccaacgacccccgcccattgacgtcaataatgacgtatgttcccatagtaacgccaatagggactttccattgacgtcaatgggtggagtatttacggtaaactgcccacttggcagtacatcaagtgtatcatatgccaagtacgccccctattgacgtcaatgacggtaaatggcccgcctggcattatgcccagtacatgaccttatgggactttcctacttggcagtacatctacgtattagtcatcgctattaccatggtgatgcggttttggcagtacatcaatgggcgtggatagcggtttgactcacggggatttccaagtctccaccccattgacgtcaatgggagtttgttttggcaccaaaatcaacgggactttccaaaatgtcgtaacaactccgccccattgacgcaaatgggcggtaggcgtgtacggtgggaggtctatataagcagagctggtttagtgaaccgtcagatccgctagcgctaccggactcagatctcgagctcaagcttcgaattctgcagtcgacggtaccgcgggcccgggatccaccggtcgccaccatggtgagcaagggcgaggagctgttcaccggggtggtgcccatcctggtcgagctggacggcgacgtaaacggccacaagttcagcgtgtccggcgagggcgagggcgatgccacctacggcaagctgaccctgaagttcatctgcaccaccggcaagctgcccgtgccctggcccaccctcgtgaccaccctgacctacggcgtgcagtgcttcagccgctaccccgaccacatgaagcagcacgacttcttcaagtccgccatgcccgaaggctacgtccaggagcgcaccatcttcttcaaggacgacggcaactacaagacccgcgccgaggtgaagttcgagggcgacaccctggtgaaccgcatcgagctgaagggcatcgacttcaaggaggacggcaacatcctggggcacaagctggagtacaactacaacagccacaacgtctatatcatggccgacaagcagaagaacggcatcaaggtgaacttcaagatccgccacaacatcgaggacggcagcgtgcagctcgccgaccactaccagcagaacacccccatcggcgacggccccgtgctgctgcccgacaaccactacctgagcacccagtccgccctgagcaaagaccccaacgagaagcgcgatcacatggtcctgctggagttcgtgaccgccgccgggatcactctcggcatggacgagctgtacaagtaaagcggccgcgactctagatcataatcagccataccacatttgtagaggttttacttgctttaaaaaacctcccacacctccccctgaacctgaaacataaaatgaatgcaattgttgttgttaacttgtttattgcagcttataatggttacaaataaagcaatagcatcacaaatttcacaaataaagcatttttttcactgc

SEQ ID NO: 2 - DNA, 3712 bp, Artificial Sequence
  2 Ambystoma laterale x Ambystoma jeffersonianum
ccatgcattagttattaatagtaatcaattacggggtcattagttcatagcccatatatggagttccgcgttacataacttacggtaaatggcccgcctggctgaccgcccaacgacccccgcccattgacgtcaataatgacgtatgttcccatagtaacgccaatagggactttccattgacgtcaatgggtggagtatttacggtaaactgcccacttggcagtacatcaagtgtatcatatgccaagtacgccccctattgacgtcaatgacggtaaatggcccgcctggcattatgcccagtacatgaccttatgggactttcctacttggcagtacatctacgtattagtcatcgctattaccatggtgatgcggttttggcagtacatcaatgggcgtggatagcggtttgactcacggggatttccaagtctccaccccattgacgtcaatgggagtttgttttggcaccaaaatcaacgggactttccaaaatgtcgtaacaactccgccccattgacgcaaatgggcggtaggcgtgtacggtgggaggtctatataagcagagctggtttagtgaaccgtcagatccgctagcgctaccggactcagatctcgagctcaagcttcgaattctgcagtcgacggtaccgcgggcccgggatccaccggtcgccaccatggtgagcaagggcgaggagctgttcaccggggtggtgcccatcctggtcgagctggacggcgacgtaaacggccacaagttcagcgtgtccggcgagggcgagggcgatgccacctacggcaagctgaccctgaagttcatctgcaccaccggcaagctgcccgtgccctggcccaccctcgtgaccaccctgacctacggcgtgcagtgcttcagccgctaccccgaccacatgaagcagcacgacttcttcaagtccgccatgcccgaaggctacgtccaggagcgcaccatcttcttcaaggacgacggcaactacaagacccgcgccgaggtgaagttcgagggcgacaccctggtgaaccgcatcgagctgaagggcatcgacttcaaggaggacggcaacatcctggggcacaagctggagtacaactacaacagccacaacgtctatatcatggccgacaagcagaagaacggcatcaaggtgaacttcaagatccgccacaacatcgaggacggcagcgtgcagctcgccgaccactaccagcagaacacccccatcggcgacggccccgtgctgctgcccgacaaccactacctgagcacccagtccgccctgagcaaagaccccaacgagaagcgcgatcacatggtcctgctggagttcgtgaccgccgccgggatcactctcggcatggacgagctgtacaagtaaagcggccgcgactctagatcataatcagccataccacatttgtagaggttttacttgctttaaaaaacctcccacacctccccctgaacctgaaacataaaatgaatgcaattgttgttgttaacttgtttattgcagcttataatggttacaaataaagcaatagcatcacaaatttcacaaataaagcatttttttcactgcccatgcattagttattaatagtaatcaattacggggtcattagttcatagcccatatatggagttccgcgttacataacttacggtaaatggcccgcctggctgaccgcccaacgacccccgcccattgacgtcaataatgacgtatgttcccatagtaacgccaatagggactttccattgacgtcaatgggtggagtatttacggtaaactgcccacttggcagtacatcaagtgtatcatatgccaagtacgccccctattgacgtcaatgacggtaaatggcccgcctggcattatgcccagtacatgaccttatgggactttcctacttggcagtacatctacgtattagtcatcgctattaccatggtgatgcggttttggcagtacatcaatgggcgtggatagcggtttgactcacggggatttccaagtctccaccccattgacgtcaatgggagtttgttttggcaccaaaatcaacgggactttccaaaatgtcgtaacaactccgccccattgacgcaaatgggcggtaggcgtgtacggtgggaggtctatataagcagagctggtttagtgaaccgtcagatccgctagcccaccatgaccgagtacaagcccacggtgcgcctcgccacccgcgacgacgtcccccgggccgtacgcaccctcgccgccgcgttcgccgactaccccgccacgcgccacaccgtcgacccggaccgccacatcgagcgggtcaccgagctgcaagaactcttcctcacgcgcgtcgggctcgacatcggcaaggtgtgggtcgcggacgacggcgccgcggtggcggtctggaccacgccggagagcgtcgaagcgggggcggtgttcgccgagatcggcccgcgcatggccgagttgagcggttcccggctggccgcgcagcaacagatggaaggcctcctggcgccgcaccggcccaaggagcccgcgtggttcctggccaccgtcggcgtctcgcccgaccaccagggcaagggtctgggcagcgccgtcgtgctccccggagtggaggcggccgagcgcgccggggtgcccgccttcctggagacctccgcgccccgcaacctccccttctacgagcggctcggcttcaccgtcaccgccgacgtcgaggtgcccgaaggaccgcgcacctggtgcatgacccgcaagcccggtgccggatcgggagagggcagaggaagtctgctaacatgcggtgacgtcgaggagaatcctggcccaccggtcgccaccatggtgagcaagggcgaggaggataacatggccatcatcaaggagttcatgcgcttcaaggtgcacatggagggctccgtgaacggccacgagttcgagatcgagggcgagggcgagggccgcccctacgagggcacccagaccgccaagctgaaggtgaccaagggtggccccctgcccttcgcctgggacatcctgtcccctcagttcatgtacggctccaaggcctacgtgaagcaccccgccgacatccccgactacttgaagctgtccttccccgagggcttcaagtgggagcgcgtgatgaacttcgaggacggcggcgtggtgaccgtgacccaggactcctccctgcaggacggcgagttcatctacaaggtgaagctgcgcggcaccaacttcccctccgacggccccgtaatgcagaagaagaccatgggctgggaggcctcctccgagcggatgtaccccgaggacggcgccctgaagggcgagatcaagcagaggctgaagctgaaggacggcggccactacgacgctgaggtcaagaccacctacaaggccaagaagcccgtgcagctgcccggcgcctacaacgtcaacatcaagttggacatcacctcccacaacgaggactacaccatcgtggaacagtacgaacgcgccgagggccgccactccaccggcggcatggacgagctgtacaagtaagaattcgtcgagggacctaataacttcgtatagcatacattatacgaagttatacatgtttaagggttccggttccactaggtacaattcgatatcaagcttatcgataa

SEQ ID NO: 3 - DNA, 28 bp, Artificial Sequence
  2 Ambystoma laterale x Ambystoma jeffersonianum
gcctttttacggttcctggccttttgct

SEQ ID NO: 4 - DNA, 28 bp, Artificial Sequence
  2 Ambystoma laterale x Ambystoma jeffersonianum
agggattttgccgatttcggcctattgg

SEQ ID NO: 5 - DNA, 2003 bp, Artificial Sequence
  2 Ambystoma laterale x Ambystoma jeffersonianum
ggactcagatctcgagctcaagcttcgaattctgcagtcgacggtaccgcgggcccgggatccaccggtcgccaccatggtgagcaagggcgaggagctgttcaccggggtggtgcccatcctggtcgagctggacggcgacgtaaacggccacaagttcagcgtgtccggcgagggcgagggcgatgccacctacggcaagctgaccctgaagttcatctgcaccaccggcaagctgcccgtgccctggcccaccctcgtgaccaccctgacctacggcgtgcagtgcttcagccgctaccccgaccacatgaagcagcacgacttcttcaagtccgccatgcccgaaggctacgtccaggagcgcaccatcttcttcaaggacgacggcaactacaagacccgcgccgaggtgaagttcgagggcgacaccctggtgaaccgcatcgagctgaagggcatcgacttcaaggaggacggcaacatcctggggcacaagctggagtacaactacaacagccacaacgtctatatcatggccgacaagcagaagaacggcatcaaggtgaacttcaagatccgccacaacatcgaggacggcagcgtgcagctcgccgaccactaccagcagaacacccccatcggcgacggccccgtgctgctgcccgacaaccactacctgagcacccagtccgccctgagcaaagaccccaacgagaagcgcgatcacatggtcctgctggagttcgtgaccgccgccgggatcactctcggcatggacgagctgtacaagtaaagcggccgcgactctagatcataatcagccataccacatttgtagaggttttacttgctttaaaaaacctcccacacctccccctgaacctgaaacataaaatgaatgcaattgttgttgttaacttgtttattgcagcttataatggttacaaataaagcaatagcatcacaaatttcacaaataaagcatttttttcactgcggatccacgcgccctgtagcggcgcattaagcgcggcgggtgtggtggttacgcgcagcgtgaccgctacacttgccagcgccctagcgcccgctcctttcgctttcttcccttcctttctcgccacgttcgccggctttccccgtcaagctctaaatcgggggctccctttagggttccgatttagtgctttacggcacctcgaccccaaaaaacttgatttgggtgatggttcacgtagtgggccatcgccctgatagacggtttttcgccctttgacgttggagtccacgttctttaatagtggactcttgttccaaactggttaacaacactcaaccctatctcgggctattcttttgatttataagggattttgccgatttcggggtaccatgcattagttattaatagtaatcaattacggggtcattagttcatagcccatatatggagttccgcgttacataacttacggtaaatggcccgcctggctgaccgcccaacgacccccgcccattgacgtcaataatgacgtatgttcccatagtaacgccaatagggactttccattgacgtcaatgggtggagtatttacggtaaactgcccacttggcagtacatcaagtgtatcatatgccaagtacgccccctattgacgtcaatgacggtaaatggcccgcctggcattatgcccagtacatgaccttatgggactttcctacttggcagtacatctacgtattagtcatcgctattaccatggtgatgcggttttggcagtacatcaatgggcgtggatagcggtttgactcacggggatttccaagtctccaccccattgacgtcaatgggagtttgttttggcaccaaaatcaacgggactttccaaaatgtcgtaacaactccgccccattgacgcaaatgggcggtaggcgtgtacggtgggaggtctatataagcagagctggtttagtgaaccgtcagatccgctagcgctacc

SEQ ID NO: 6 - DNA, 4105 bp, Artificial Sequence
  2 Ambystoma laterale x Ambystoma jeffersonianum
aacaacactcaaccctatctcgggctattcttttgatttataagggattttgccgatttcggggtaccatgcattagttattaatagtaatcaattacggggtcattagttcatagcccatatatggagttccgcgttacataacttacggtaaatggcccgcctggctgaccgcccaacgacccccgcccattgacgtcaataatgacgtatgttcccatagtaacgccaatagggactttccattgacgtcaatgggtggagtatttacggtaaactgcccacttggcagtacatcaagtgtatcatatgccaagtacgccccctattgacgtcaatgacggtaaatggcccgcctggcattatgcccagtacatgaccttatgggactttcctacttggcagtacatctacgtattagtcatcgctattaccatggtgatgcggttttggcagtacatcaatgggcgtggatagcggtttgactcacggggatttccaagtctccaccccattgacgtcaatgggagtttgttttggcaccaaaatcaacgggactttccaaaatgtcgtaacaactccgccccattgacgcaaatgggcggtaggcgtgtacggtgggaggtctatataagcagagctggtttagtgaaccgtcagatccgctagcgctaccggactcagatctcgagctcaagcttcgaattctgcagtcgacggtaccgcgggcccgggatccaccggtcgccaccatggtgagcaagggcgaggagctgttcaccggggtggtgcccatcctggtcgagctggacggcgacgtaaacggccacaagttcagcgtgtccggcgagggcgagggcgatgccacctacggcaagctgaccctgaagttcatctgcaccaccggcaagctgcccgtgccctggcccaccctcgtgaccaccctgacctacggcgtgcagtgcttcagccgctaccccgaccacatgaagcagcacgacttcttcaagtccgccatgcccgaaggctacgtccaggagcgcaccatcttcttcaaggacgacggcaactacaagacccgcgccgaggtgaagttcgagggcgacaccctggtgaaccgcatcgagctgaagggcatcgacttcaaggaggacggcaacatcctggggcacaagctggagtacaactacaacagccacaacgtctatatcatggccgacaagcagaagaacggcatcaaggtgaacttcaagatccgccacaacatcgaggacggcagcgtgcagctcgccgaccactaccagcagaacacccccatcggcgacggccccgtgctgctgcccgacaaccactacctgagcacccagtccgccctgagcaaagaccccaacgagaagcgcgatcacatggtcctgctggagttcgtgaccgccgccgggatcactctcggcatggacgagctgtacaagtaaagcggccgcgactctagatcataatcagccataccacatttgtagaggttttacttgctttaaaaaacctcccacacctccccctgaacctgaaacataaaatgaatgcaattgttgttgttaacttgtttattgcagcttataatggttacaaataaagcaatagcatcacaaatttcacaaataaagcatttttttcactgcccatgcattagttattaatagtaatcaattacggggtcattagttcatagcccatatatggagttccgcgttacataacttacggtaaatggcccgcctggctgaccgcccaacgacccccgcccattgacgtcaataatgacgtatgttcccatagtaacgccaatagggactttccattgacgtcaatgggtggagtatttacggtaaactgcccacttggcagtacatcaagtgtatcatatgccaagtacgccccctattgacgtcaatgacggtaaatggcccgcctggcattatgcccagtacatgaccttatgggactttcctacttggcagtacatctacgtattagtcatcgctattaccatggtgatgcggttttggcagtacatcaatgggcgtggatagcggtttgactcacggggatttccaagtctccaccccattgacgtcaatgggagtttgttttggcaccaaaatcaacgggactttccaaaatgtcgtaacaactccgccccattgacgcaaatgggcggtaggcgtgtacggtgggaggtctatataagcagagctggtttagtgaaccgtcagatccgctagcccaccatgaccgagtacaagcccacggtgcgcctcgccacccgcgacgacgtcccccgggccgtacgcaccctcgccgccgcgttcgccgactaccccgccacgcgccacaccgtcgacccggaccgccacatcgagcgggtcaccgagctgcaagaactcttcctcacgcgcgtcgggctcgacatcggcaaggtgtgggtcgcggacgacggcgccgcggtggcggtctggaccacgccggagagcgtcgaagcgggggcggtgttcgccgagatcggcccgcgcatggccgagttgagcggttcccggctggccgcgcagcaacagatggaaggcctcctggcgccgcaccggcccaaggagcccgcgtggttcctggccaccgtcggcgtctcgcccgaccaccagggcaagggtctgggcagcgccgtcgtgctccccggagtggaggcggccgagcgcgccggggtgcccgccttcctggagacctccgcgccccgcaacctccccttctacgagcggctcggcttcaccgtcaccgccgacgtcgaggtgcccgaaggaccgcgcacctggtgcatgacccgcaagcccggtgccggatcgggagagggcagaggaagtctgctaacatgcggtgacgtcgaggagaatcctggcccaccggtcgccaccatggtgagcaagggcgaggaggataacatggccatcatcaaggagttcatgcgcttcaaggtgcacatggagggctccgtgaacggccacgagttcgagatcgagggcgagggcgagggccgcccctacgagggcacccagaccgccaagctgaaggtgaccaagggtggccccctgcccttcgcctgggacatcctgtcccctcagttcatgtacggctccaaggcctacgtgaagcaccccgccgacatccccgactacttgaagctgtccttccccgagggcttcaagtgggagcgcgtgatgaacttcgaggacggcggcgtggtgaccgtgacccaggactcctccctgcaggacggcgagttcatctacaaggtgaagctgcgcggcaccaacttcccctccgacggccccgtaatgcagaagaagaccatgggctgggaggcctcctccgagcggatgtaccccgaggacggcgccctgaagggcgagatcaagcagaggctgaagctgaaggacggcggccactacgacgctgaggtcaagaccacctacaaggccaagaagcccgtgcagctgcccggcgcctacaacgtcaacatcaagttggacatcacctcccacaacgaggactacaccatcgtggaacagtacgaacgcgccgagggccgccactccaccggcggcatggacgagctgtacaagtaagaattcgtcgagggacctaataacttcgtatagcatacattatacgaagttatacatgtttaagggttccggttccactaggtacaattcgatatcaagcttatcgataaggatccacgcgccctgtagcggcgcattaagcgcggcgggtgtggtggttacgcgcagcgtgaccgctacacttgccagcgccctagcgcccgctcctttcgctttcttcccttcctttctcgccacgttcgccggctttccccgtcaagctctaaatcgggggctccctttagggttccgatttagtgctttacggcacctcgaccccaaaaaacttgatttgggtgatggttcacgtagtgggccatcgccctgatagacggtttttcgccctttgacgttggagtccacgttctttaatagtggactcttgttccaaactggtt

SEQ ID NO: 7 - DNA, 2003 bp, Artificial Sequence
  2 Ambystoma laterale x Ambystoma jeffersonianum
gcagtgaaaaaaatgctttatttgtgaaatttgtgatgctattgctttatttgtaaccattataagctgcaataaacaagttaacaacaacaattgcattcattttatgtttcaggttcagggggaggtgtgggaggttttttaaagcaagtaaaacctctacaaatgtggtatggctgattatgatctagagtcgcggccgctttacttgtacagctcgtccatgccgagagtgatcccggcggcggtcacgaactccagcaggaccatgtgatcgcgcttctcgttggggtctttgctcagggcggactgggtgctcaggtagtggttgtcgggcagcagcacggggccgtcgccgatgggggtgttctgctggtagtggtcggcgagctgcacgctgccgtcctcgatgttgtggcggatcttgaagttcaccttgatgccgttcttctgcttgtcggccatgatatagacgttgtggctgttgtagttgtactccagcttgtgccccaggatgttgccgtcctccttgaagtcgatgcccttcagctcgatgcggttcaccagggtgtcgccctcgaacttcacctcggcgcgggtcttgtagttgccgtcgtccttgaagaagatggtgcgctcctggacgtagccttcgggcatggcggacttgaagaagtcgtgctgcttcatgtggtcggggtagcggctgaagcactgcacgccgtaggtcagggtggtcacgagggtgggccagggcacgggcagcttgccggtggtgcagatgaacttcagggtcagcttgccgtaggtggcatcgccctcgccctcgccggacacgctgaacttgtggccgtttacgtcgccgtccagctcgaccaggatgggcaccaccccggtgaacagctcctcgcccttgctcaccatggtggcgaccggtggatcccgggcccgcggtaccgtcgactgcagaattcgaagcttgagctcgagatctgagtccggtagcgctagcggatctgacggttcactaaaccagctctgcttatatagacctcccaccgtacacgcctaccgcccatttgcgtcaatggggcggagttgttacgacattttggaaagtcccgttgattttggtgccaaaacaaactcccattgacgtcaatggggtggagacttggaaatccccgtgagtcaaaccgctatccacgcccattgatgtactgccaaaaccgcatcaccatggtaatagcgatgactaatacgtagatgtactgccaagtaggaaagtcccataaggtcatgtactgggcataatgccaggcgggccatttaccgtcattgacgtcaatagggggcgtacttggcatatgatacacttgatgtactgccaagtgggcagtttaccgtaaatactccacccattgacgtcaatggaaagtccctattggcgttactatgggaacatacgtcattattgacgtcaatgggcgggggtcgttgggcggtcagccaggcgggccatttaccgtaagttatgtaacgcggaactccatatatgggctatgaactaatgaccccgtaattgattactattaataactaatgcatggggatccacgcgccctgtagcggcgcattaagcgcggcgggtgtggtggttacgcgcagcgtgaccgctacacttgccagcgccctagcgcccgctcctttcgctttcttcccttcctttctcgccacgttcgccggctttccccgtcaagctctaaatcgggggctccctttagggttccgatttagtgctttacggcacctcgaccccaaaaaacttgatttgggtgatggttcacgtagtgggccatcgccctgatagacggtttttcgccctttgacgttggagtccacgttctttaatagtggactcttgttccaaactggttaacaacactcaaccctatctcgggctattcttttgatttataagggattttgccgatttcggggta